European Patent Application EP 4 163 301 A1, published April 12, 2023. Title: Humanized anti-GPC-1 antibody. Applicant: Kouchi University. The sequence listing filed with the application follows.

SEQUENCE LISTING (92 sequences)

SEQ ID NO: 1 - DNA, 1677 bp, Homo sapiens
atggagctccgggcccgaggctggtggctgctatgtgcggccgcagcgctggtcgcctgcgcccgcggggacccggccagcaagagccggagctgcggcgaggtccgccagatctacggagccaagggcttcagcctgagcgacgtgccccaggcggagatctcgggtgagcacctgcggatctgtccccagggctacacctgctgcaccagcgagatggaggagaacctggccaaccgcagccatgccgagctggagaccgcgctccgggacagcagccgcgtcctgcaggccatgcttgccacccagctgcgcagcttcgatgaccacttccagcacctgctgaacgactcggagcggacgctgcaggccaccttccccggcgccttcggagagctgtacacgcagaacgcgagggccttccgggacctgtactcagagctgcgcctgtactaccgcggtgccaacctgcacctggaggagacgctggccgagttctgggcccgcctgctcgagcgcctcttcaagcagctgcacccccagctgctgctgcctgatgactacctggactgcctgggcaagcaggccgaggcgctgcggcccttcggggaggccccgagagagctgcgcctgcgggccacccgtgccttcgtggctgctcgctcctttgtgcagggcctgggcgtggccagcgacgtggtccggaaagtggctcaggtccccctgggcccggagtgctcgagagctgtcatgaagctggtctactgtgctcactgcctgggagtccccggcgccaggccctgccctgactattgccgaaatgtgctcaagggctgccttgccaaccaggccgacctggacgccgagtggaggaacctcctggactccatggtgctcatcaccgacaagttctggggtacatcgggtgtggagagtgtcatcggcagcgtgcacacgtggctggcggaggccatcaacgccctccaggacaacagggacacgctcacggccaaggtcatccagggctgcgggaaccccaaggtcaacccccagggccccgggcctgaggagaagcggcgccggggcaagctggccccgcgggagaggccaccttcaggcacgctggagaagctggtctccgaagccaaggcccagctccgcgacgtccaggacttctggatcagcctcccagggacactgtgcagtgagaagatggccctgagcactgccagtgatgaccgctgctggaacgggatggccagaggccggtacctccccgaggtcatgggtgacggcctggccaaccagatcaacaaccccgaggtggaggtggacatcaccaagccggacatgaccatccggcagcagatcatgcagctgaagatcatgaccaaccggctgcgcagcgcctacaacggcaacgacgtggacttccaggacgccagtgacgacggcagcggctcgggcagcggtgatggctgtctggatgacctctgcagccggaaggtcagcaggaagagctccagctcccggacgcccttgacccatgccctcccaggcctgtcagagcaggaaggacagaagacctcggctgccagctgcccccagcccccgaccttcctcctgcccctcctcctcttcctggcccttacagtagccaggccccggtggcggtaa

SEQ ID NO: 2 - protein, 558 aa, Homo sapiens
MELRARGWWLLCAAAALVACARGDPASKSRSCGEVRQIYGAKGFSLSDVPQAEISGEHLRICPQGYTCCTSEMEENLANRSHAELETALRDSSRVLQAMLATQLRSFDDHFQHLLNDSERTLQATFPGAFGELYTQNARAFRDLYSELRLYYRGANLHLEETLAEFWARLLERLFKQLHPQLLLPDDYLDCLGKQAEALRPFGEAPRELRLRATRAFVAARSFVQGLGVASDVVRKVAQVPLGPECSRAVMKLVYCAHCLGVPGARPCPDYCRNVLKGCLANQADLDAEWRNLLDSMVLITDKFWGTSGVESVIGSVHTWLAEAINALQDNRDTLTAKVIQGCGNPKVNPQGPGPEEKRRRGKLAPRERPPSGTLEKLVSEAKAQLRDVQDFWISLPGTLCSEKMALSTASDDRCWNGMARGRYLPEVMGDGLANQINNPEVEVDITKPDMTIRQQIMQLKIMTNRLRSAYNGNDVDFQDASDDGSGSGSGDGCLDDLCSRKVSRKSSSSRTPLTHALPGLSEQEGQKTSAASCPQPPTFLLPLLLFLALTVARPRWR

SEQ ID NO: 3 - DNA, 1673 bp, Mus musculus
tggaactccggacccgaggctggtggctgctgtgcgcggccgccgcgctggtcgtctgcgcccgcggggaccccgccagcaagagccggagctgcagcgaagtccgccagatctacggggctaagggctttagcctgagcgatgtgcctcaggcagagatctcgggtgagcacctgcggatctgcccccagggctacacttgctgtactagtgagatggaggagaatttggccaaccacagccgaatggagctggagagcgcactccatgacagcagccgcgccctgcaggccacactggccacccagctgcatggcatcgatgaccacttccagcgcctgctgaatgactcggagcgcacactgcaggaggctttccctggggcctttggggacctgtatacgcagaacactcgtgccttccgggacctatatgctgagctgcgcctctactaccgtggggccaacctgcaccttgaggagacgctggccgagttctgggcacggctgctggagcgcctcttcaagcagctgcacccccagctgctgcctgatgactacctggactgcctgggcaagcaggcggaggcactgcggccgtttggagatgcccctcgagaactgcgcctgcgggccacccgtgcctttgtggctgcacgttcctttgtgcagggcctgggtgtggccagtgatgtagtccggaaggtggcccaggtacctctggccccagaatgttctcgggccatcatgaagttggtctactgtgctcattgccggggagtcccgggcgcccggccctgccccgactattgccgaaatgtgctcaaaggctgccttgccaaccaggccgacctggatgccgagtggaggaacctcctggactccatggtgctcatcactgacaagttctggggcccgtcgggtgcggagagtgtcattggcggtgtgcacgtgtggctggcggaggccatcaacgccctccaggacaacaaggacacactcacagctaaggtcatccaggcctgtggaaaccccaaggtcaatccccacggctctgggcccgaggagaagcgtcgccgtggcaaattggcactgcaggagaagccctccacaggtactctggaaaaactggtctctgaggccaaggcccagctccgagacattcaggacttctggatcagcctcccagggacactgtgcagtgagaagatggccatgagtcctgccagtgacgaccgctgctggaatggaatttccaagggccggtacctaccagaggtgatgggtgacgggctggccaaccagatcaacaaccctgaggtggaagtggacatcaccaagccagacatgaccatccgccagcagattatgcagctcaagatcatgaccaaccgtttacgtggcgcctatggcggcaacgacgtggacttccaggatgctagtgatgacggcagtggctccggcagcggtggcggatgcccagatgacacctgtggccggagggtcagcaagaagagttccagctcccggacccccttgacccatgccctccccggcctgtcagaacaggagggacagaagacctcagctgccacctgcccagagccccacagcttcttcctgctcttcctcgtcaccttggtccttgcggcagccaggcccaggtggcggtaa

SEQ ID NO: 4 - protein, 557 aa, Mus musculus
MELRTRGWWLLCAAAALVVCARGDPASKSRSCSEVRQIYGAKGFSLSDVPQAEISGEHLRICPQGYTCCTSEMEENLANHSRMELESALHDSSRALQATLATQLHGIDDHFQRLLNDSERTLQEAFPGAFGDLYTQNTRAFRDLYAELRLYYRGANLHLEETLAEFWARLLERLFKQLHPQLLPDDYLDCLGKQAEALRPFGDAPRELRLRATRAFVAARSFVQGLGVASDVVRKVAQVPLAPECSRAIMKLVYCAHCRGVPGARPCPDYCRNVLKGCLANQADLDAEWRNLLDSMVLITDKFWGPSGAESVIGGVHVWLAEAINALQDNKDTLTAKVIQACGNPKVNPHGSGPEEKRRRGKLALQEKPSTGTLEKLVSEAKAQLRDIQDFWISLPGTLCSEKMAMSPASDDRCWNGISKGRYLPEVMGDGLANQINNPEVEVDITKPDMTIRQQIMQLKIMTNRLRGAYGGNDVDFQDASDDGSGSGSGGGCPDDTCGRRVSKKSSSSRTPLTHALPGLSEQEGQKTSAATCPEPHSFFLLFLVTLVLAAARPRWR

SEQ ID NO: 5 - protein, 119 aa, artificial sequence
  01a033 heavy chain variable region
QVQLKQSGPELVKPGASVKISCKASGYSFTGYYMHWVKQSPEKSLEWIGEINPSTGDTTYNQKFKAKATLTVDKSSSTAYMQLKSLTSEDSAVYYCAREKRDDGVFAYWGQGTLVTVSS

SEQ ID NO: 6 - protein, 107 aa, artificial sequence
  01a033 light chain variable region
DIVMSQSPKSMSMSVGERVALSCKASENVGTYVSWYQQKPEQSPKLLIYGASNRYTGVPDRFTGSGSATDFTLTISSVQAEDLADYYCGQSYSYPLTFGAGTKLELK

SEQ ID NO: 7 - protein, 119 aa, artificial sequence
  humanized heavy chain variable region
QVQLVQSGAEVKKPGASVKVSCKASGYTFTGYYMHWVRQAPGQGLEWMGEINPSTGDTTYNQKFKARVTMTRDTSTSTVYMELSSLRSEDTAVYYCAREKRDDGVFAYWGQGTLVTVSS

SEQ ID NO: 8 - protein, 108 aa, artificial sequence
  T2 humanized light chain variable region
DIVMTQSPSFLSASVGDRVTITCRASQGISSYLVWYQQKPGKPPKLLIYSASVLQSGVPSRFSGRGYGTDFTLTISSLQPEDFATYYCQQSFSIPPVTFGGGTKVEIK

SEQ ID NO: 9 - protein, 107 aa, artificial sequence
  T7 humanized light chain variable region
AIQLTQSPSTLSASVGDRVTITCRASQSISSWLAWYQQKPGKAPKLLISDASNLASGVPLRFSGSGFGTHFTLTIDNLQPEDIATYSCQQYNNYPFTFGLGTKLEIK

SEQ ID NO: 10 - protein, 107 aa, artificial sequence
  T8 humanized light chain variable region
EIVMTQSPSSVSASVGDRVTITCRTSQSISSYLNWYQLRPGRAPKLLIYAASNLQSGVPSRFSGSGFGTDFTLTISSVQPEDFATYYCQQAKSYPLTFGGGTKVDIK

SEQ ID NO: 11 - protein, 108 aa, artificial sequence
  T1 humanized light chain variable region
DIVMTQSPSFLSASVGDRVTITCRASQGISSYLVWYQQKPGKAPKLLIYSASVLQSGVPSRFSGRGYGTDFTLTISSLQPEDFATYYCQQSFSIPPVTFGGGTKVEIK

SEQ ID NO: 12 - protein, 107 aa, artificial sequence
  T36 humanized light chain variable region
NIQMTQSPSSLSASVGDRVTITCQASQDISNYLNWYQQRPGKAPQLLIYGASNLERGVPSRFSGSGFGTDFTLTISSVQPEDFATYYCQQAKSYPLTFGGGTKVEIK

SEQ ID NO: 13 - protein, 107 aa, artificial sequence
  T57 humanized light chain variable region
EIVMTQSPSSLSASVGDRVTISCRTSQTIRHYLNWYQQKPGKAPKLLIYDASNLKTGVPSRFSGSGSGTSFTLTISSLQPDDFATYYCQQSYSTPRTFGQGTKVEIK

SEQ ID NO: 14 - protein, 107 aa, artificial sequence
  T10 humanized light chain variable region
EIVLTQSPSTLSASVGDRVTITCRASQSISSWLAWYQQIPGKAPRILISSASILQSGAPSRFSGSGFGTDFTLTISSVQPEDFATYYCQQAKSYPLTFGGGTKLEIK

SEQ ID NO: 15 - protein, 107 aa, artificial sequence
  T34 humanized light chain variable region
VIWMTQSPSSVSASVGDRVTITCRASQAINGWLAWYQQKPGKAPRILIYSASTLQTGAPSRFSGSGFGTDFTLTISSVQPEDFATYYCQQAKSYPLTFGGGTKVEIK

SEQ ID NO: 16 - protein, 107 aa, artificial sequence
  T56 humanized light chain variable region
DIVMTQSPSTLSASVGDRVTIICRASQSIGPWLAWYQQKSGKAPKLLIYGASNLQSGVPSRFSGSGYGTDFTLTISSLQPEDFATYYCQQTSSAPFTFGPGTKVDIK

SEQ ID NO: 17 - protein, 107 aa, artificial sequence
  T3 humanized light chain variable region
DIVMTQSPSSVSASVGDRVSITCRASEHINGWLAWYQQIPGKAPRILISSASILQSGAPSRFSGSGFGTDFTLTISSVQPEDFATYYCQQAKSYPLTFGGGTKVEIK

SEQ ID NO: 18 - protein, 107 aa, artificial sequence
  T11 humanized light chain variable region
AIRMTQSPSSLSASVGDRVTITCRASRSISTYLHWYQQKAGKAPKLLIYSAYNLQSGVPSRFSGSGSGTDFTLTISSLQPEDFATYYCQQSYSTPYTFGQGTKVEIK

SEQ ID NO: 19 - protein, 107 aa, artificial sequence
  T28 humanized light chain variable region
DIQMTQSPSSLSASLGEMVTITCRASESIHSYLNWYQQKPGKAPNLLIYDASNLESGVPSRFSGSGYGTDFTLTISSLQPEDFATYYCQQSYGPPITFGQGTRLEIK

SEQ ID NO: 20 - protein, 107 aa, artificial sequence
  T43 humanized light chain variable region
DIVMTQSPSSLSASVGDRVTITCRASQGIRSALAWYQQKPGKAPKLLIYDASNLQSGVPSRFSGSGSGTDFTLTISDVQAEDFGTYYCQQSFGPPRTFGQGTRLEIK

SEQ ID NO: 21 - protein, 107 aa, artificial sequence
  T59 humanized light chain variable region
EIVMTQSPSSLSASVGDRVTITCQASQHISNKLNWYQQKPGKAPKLLIYDASNLETGVPSRFSGSGYGTDFTFTVSSLQPEDIATYYCQQYDNLPITFGQGTRLEIK

SEQ ID NO: 22 - protein, 107 aa, artificial sequence
  T31 humanized light chain variable region
AIQMTQSPATLSLSPGQRATLSCRASQSVSNYLAWYQQKPGQAPRLLIYDVSNRASGIPARFSGSGSGTDFTLTISSLEPEDFAIYYCQQRSNWPLTFGQGTKVDIK

SEQ ID NO: 23 - protein, 107 aa, artificial sequence
  T22 humanized light chain variable region
AIQMTQSPASLSASLGDRITITCRTSQTVAGYLNWYQQTPGNAPKLLIYSASNLQSGVPSRFSGSGSGRDFSLTISSLQSEDSATYYCQHSYSTPYTFGQGTKVEIK

SEQ ID NO: 24 - protein, 107 aa, artificial sequence
  T26 humanized light chain variable region
DVVMTQSPSSLSASVGERVTITCRASQSISSYLNWYQQKPGKAPKLLIYAASSRATGIPHRYSGSGSGTVFTLTISRLEPEDFATYYCQQFHSYPITFGQGTRLEIK

SEQ ID NO: 25 - protein, 107 aa, artificial sequence
  T32 humanized light chain variable region
DVVMTQSPGTLSLSPGERATLSCSASQSVSSNLAWYQQKPGQAPRLLIYGTSSRATGVPARFSGSGSGTEFTLTISSLQSEDFAAYYCQQYNSWPLTFGGGTKVEIK

SEQ ID NO: 26 - protein, 108 aa, artificial sequence
  T33 humanized light chain variable region
DVVMTQSPATLSVPPGDRATLSCRASQSVSSRLAWYQQKPGQAPKLLIYGASTRATGIPARFSGSWSGTEFTLTVSSLQSEDSAVYYCQQYNDWPRYTFGQGTKLEIK

SEQ ID NO: 27 - protein, 107 aa, artificial sequence
  T29 humanized light chain variable region
DIVMTQSPSSLSASVGDRVTITCRASQDISSYLNWYQQKPGEAPKLLVYGASNLQRGVPPGFRGSGSGTDFTLTINNLQPEDFATYYCQQSSTSPITFGQGTRLEIK

SEQ ID NO: 28 - protein, 5 aa, artificial sequence
  humanized heavy chain CDR1
GYYMH

SEQ ID NO: 29 - protein, 16 aa, artificial sequence
  humanized heavy chain CDR2
EINPSTGDTTYNQKFK

SEQ ID NO: 30 - protein, 10 aa, artificial sequence
  humanized heavy chain CDR3
EKRDDGVFAY

SEQ ID NO: 31 - protein, 11 aa, artificial sequence
  T2 light chain CDR1
RASQGISSYLV

SEQ ID NO: 32 - protein, 7 aa, artificial sequence
  T2 light chain CDR2
SASVLQS

SEQ ID NO: 33 - protein, 10 aa, artificial sequence
  T2 light chain CDR3
QQSFSIPPVT

SEQ ID NO: 34 - protein, 11 aa, artificial sequence
  T7 light chain CDR1
RASQSISSWLA

SEQ ID NO: 35 - protein, 7 aa, artificial sequence
  T7 light chain CDR2
DASNLAS

SEQ ID NO: 36 - protein, 9 aa, artificial sequence
  T7 light chain CDR3
QQYNNYPFT

SEQ ID NO: 37 - protein, 11 aa, artificial sequence
  T8 light chain CDR1
RTSQSISSYLN

SEQ ID NO: 38 - protein, 7 aa, artificial sequence
  T8 light chain CDR2
AASNLQS

SEQ ID NO: 39 - protein, 9 aa, artificial sequence
  T8 light chain CDR3
QQAKSYPLT

SEQ ID NO: 40 - protein, 11 aa, artificial sequence
  T1 light chain CDR1
RASQGISSYLV

SEQ ID NO: 41 - protein, 7 aa, artificial sequence
  T1 light chain CDR2
SASVLQS

SEQ ID NO: 42 - protein, 10 aa, artificial sequence
  T1 light chain CDR3
QQSFSIPPVT

SEQ ID NO: 43 - protein, 11 aa, artificial sequence
  T36 light chain CDR1
QASQDISNYLN

SEQ ID NO: 44 - protein, 7 aa, artificial sequence
  T36 light chain CDR2
GASNLER

SEQ ID NO: 45 - protein, 9 aa, artificial sequence
  T36 light chain CDR3
QQAKSYPLT

SEQ ID NO: 46 - protein, 11 aa, artificial sequence
  T57 light chain CDR1
RTSQTIRHYLN

SEQ ID NO: 47 - protein, 7 aa, artificial sequence
  T57 light chain CDR2
DASNLKT

SEQ ID NO: 48 - protein, 9 aa, artificial sequence
  T57 light chain CDR3
QQSYSTPRT

SEQ ID NO: 49 - protein, 11 aa, artificial sequence
  T10 light chain CDR1
RASQSISSWLA

SEQ ID NO: 50 - protein, 7 aa, artificial sequence
  T10 light chain CDR2
SASILQS

SEQ ID NO: 51 - protein, 9 aa, artificial sequence
  T10 light chain CDR3
QQAKSYPLT

SEQ ID NO: 52 - protein, 11 aa, artificial sequence
  T34 light chain CDR1
RASQAINGWLA

SEQ ID NO: 53 - protein, 7 aa, artificial sequence
  T34 light chain CDR2
SASTLQT

SEQ ID NO: 54 - protein, 9 aa, artificial sequence
  T34 light chain CDR3
QQAKSYPLT

SEQ ID NO: 55 - protein, 11 aa, artificial sequence
  T56 light chain CDR1
RASQSIGPWLA

SEQ ID NO: 56 - protein, 7 aa, artificial sequence
  T56 light chain CDR2
GASNLQS

SEQ ID NO: 57 - protein, 9 aa, artificial sequence
  T56 light chain CDR3
QQTSSAPFT

SEQ ID NO: 58 - protein, 11 aa, artificial sequence
  T3 light chain CDR1
RASEHINGWLA

SEQ ID NO: 59 - protein, 7 aa, artificial sequence
  T3 light chain CDR2
SASILQS

SEQ ID NO: 60 - protein, 9 aa, artificial sequence
  T3 light chain CDR3
QQAKSYPLT

SEQ ID NO: 61 - protein, 11 aa, artificial sequence
  T11 light chain CDR1
RASRSISTYLH

SEQ ID NO: 62 - protein, 7 aa, artificial sequence
  T11 light chain CDR2
SAYNLQS

SEQ ID NO: 63 - protein, 9 aa, artificial sequence
  T11 light chain CDR3
QQSYSTPYT

SEQ ID NO: 64 - protein, 11 aa, artificial sequence
  T28 light chain CDR1
RASESIHSYLN

SEQ ID NO: 65 - protein, 7 aa, artificial sequence
  T28 light chain CDR2
DASNLES

SEQ ID NO: 66 - protein, 9 aa, artificial sequence
  T28 light chain CDR3
QQSYGPPIT

SEQ ID NO: 67 - protein, 11 aa, artificial sequence
  T43 light chain CDR1
RASQGIRSALA

SEQ ID NO: 68 - protein, 7 aa, artificial sequence
  T43 light chain CDR2
DASNLQS

SEQ ID NO: 69 - protein, 9 aa, artificial sequence
  T43 light chain CDR3
QQSFGPPRT

SEQ ID NO: 70 - protein, 11 aa, artificial sequence
  T59 light chain CDR1
QASQHISNKLN

SEQ ID NO: 71 - protein, 7 aa, artificial sequence
  T59 light chain CDR2
DASNLET

SEQ ID NO: 72 - protein, 9 aa, artificial sequence
  T59 light chain CDR3
QQYDNLPIT

SEQ ID NO: 73 - protein, 11 aa, artificial sequence
  T31 light chain CDR1
RASQSVSNYLA

SEQ ID NO: 74 - protein, 7 aa, artificial sequence
  T31 light chain CDR2
DVSNRAS

SEQ ID NO: 75 - protein, 9 aa, artificial sequence
  T31 light chain CDR3
QQRSNWPLT

SEQ ID NO: 76 - protein, 11 aa, artificial sequence
  T22 light chain CDR1
RTSQTVAGYLN

SEQ ID NO: 77 - protein, 7 aa, artificial sequence
  T22 light chain CDR2
SASNLQS

SEQ ID NO: 78 - protein, 9 aa, artificial sequence
  T22 light chain CDR3
QHSYSTPYT

SEQ ID NO: 79 - protein, 11 aa, artificial sequence
  T26 light chain CDR1
RASQSISSYLN

SEQ ID NO: 80 - protein, 7 aa, artificial sequence
  T26 light chain CDR1
AASSRAT

SEQ ID NO: 81 - protein, 9 aa, artificial sequence
  T26 light chain CDR3
QQFHSYPIT

SEQ ID NO: 82 - protein, 11 aa, artificial sequence
  T32 light chain CDR1
SASQSVSSNLA

SEQ ID NO: 83 - protein, 7 aa, artificial sequence
  T32 light chain CDR2
GTSSRAT

SEQ ID NO: 84 - protein, 9 aa, artificial sequence
  T32 light chain CDR3
QQYNSWPLT

SEQ ID NO: 85 - protein, 11 aa, artificial sequence
  T33 light chain CDR1
RASQSVSSRLA

SEQ ID NO: 86 - protein, 7 aa, artificial sequence
  T33 light chain CDR2
GASTRAT

SEQ ID NO: 87 - protein, 10 aa, artificial sequence
  T33 light chain CDR3
QQYNDWPRYT

SEQ ID NO: 88 - protein, 11 aa, artificial sequence
  T29 light chain CDR1
RASQDISSYLN

SEQ ID NO: 89 - protein, 7 aa, artificial sequence
  T29 light chain CDR2
GASNLQR

SEQ ID NO: 90 - protein, 9 aa, artificial sequence
  T29 light chain CDR3
QQSSTSPIT

SEQ ID NO: 91 - protein, 327 aa, artificial sequence
  heavy chain constant region of chimeric and humanized antibody
ASTKGPSVFPLAPCSRSTSESTAALGCLVKDYFPEPVTVSWNSGALTSGVHTFPAVLQSSGLYSLSSVVTVPSSSLGTKTYTCNVDHKPSNTKVDKRVESKYGPPCPPCPAPEFLGGPSVFLFPPKPKDTLMISRTPEVTCVVVDVSQEDPEVQFNWYVDGVEVHNAKTKPREEQFNSTYRVVSVLTVLHQDWLNGKEYKCKVSNKGLPSSIEKTISKAKGQPREPQVYTLPPSQEEMTKNQVSLTCLVKGFYPSDIAVEWESNGQPENNYKTTPPVLDSDGSFFLYSRLTVDKSRWQEGNVFSCSVMHEALHNHYTQKSLSLSLGK

SEQ ID NO: 92 - protein, 107 aa, artificial sequence [sequence omitted]